European Patent Application EP 4 410 815 A1, published August 7, 2024. Title: Peptide having hair loss preventing activity or hair growth promoting activity and use thereof. Applicant: CAREGENE CO., LTD. The sequence listing filed with the application follows.

SEQUENCE LISTING (17 sequences)

SEQ ID NO: 1 - protein, 9 aa, synthetic construct
CPRHFNPVC

SEQ ID NO: 2 - DNA, 20 bp, synthetic construct
  source 1..20: mol_type = other DNA
ccagctattgtaacacctca

SEQ ID NO: 3 - DNA, 20 bp, synthetic construct
  source 1..20: mol_type = other DNA
ttcagatgtaggcagctgtc

SEQ ID NO: 4 - DNA, 25 bp, synthetic construct
  source 1..25: mol_type = other DNA
accagcagcgactctgaggaggaac

SEQ ID NO: 5 - DNA, 26 bp, synthetic construct
  source 1..26: mol_type = other DNA
tgaccctcttggcagcaggatagtcc

SEQ ID NO: 6 - DNA, 28 bp, synthetic construct
  source 1..28: mol_type = other DNA
accttcgttgccctctgtgccacagatg

SEQ ID NO: 7 - DNA, 21 bp, synthetic construct
  source 1..21: mol_type = other DNA
aggcccggaggcagtccgggt

SEQ ID NO: 8 - DNA, 20 bp, synthetic construct
  source 1..20: mol_type = other DNA
ggagccaaaagggtcatcat

SEQ ID NO: 9 - DNA, 20 bp, synthetic construct
  source 1..20: mol_type = other DNA
gtgatggcatggactgtggt

SEQ ID NO: 10 - DNA, 20 bp, synthetic construct
  source 1..20: mol_type = other DNA
gatcatcgagctgagacgca

SEQ ID NO: 11 - DNA, 20 bp, synthetic construct
  source 1..20: mol_type = other DNA
ctggccccagggtatctagt

SEQ ID NO: 12 - DNA, 20 bp, synthetic construct
  source 1..20: mol_type = other DNA
ccaaatccgcaccaaggtca

SEQ ID NO: 13 - DNA, 21 bp, synthetic construct
  source 1..21: mol_type = other DNA
gtattgattgccaggaggggg

SEQ ID NO: 14 - DNA, 20 bp, synthetic construct
  source 1..20: mol_type = other DNA
cgcggcgtatccgtgtcctc

SEQ ID NO: 15 - DNA, 24 bp, synthetic construct
  source 1..24: mol_type = other DNA
agcctgttccgtctcaaacttggt

SEQ ID NO: 16 - DNA, 20 bp, synthetic construct
  source 1..20: mol_type = other DNA
cggtcaagtcggaaaattca

SEQ ID NO: 17 - DNA, 20 bp, synthetic construct
  source 1..20: mol_type = other DNA
gaggagctgggatgtggtaa